European Patent Specification EP 3 583 214 B1, published November 22, 2023. Title: METHODS AND COMPOSITIONS FOR IDENTIFYING OR QUANTIFYING TARGETS IN A BIOLOGICAL SAMPLE. Applicant: New York Genome Center. The sequence listing filed with the application follows.

SEQUENCE LISTING (39 sequences)

SEQ ID NO: 1 - DNA, 78 bp, Artificial Sequence
  Synthetic reagent sequence for analytic procedure
  misc_feature (41)..(42): n is a or g or c or t/u
gtctcgtgggctcggagatgtgtataagagacaggccaatnnbaaaaaaaaaaaaaaaaaaaaaaaaaaaaaaaaaaa

SEQ ID NO: 2 - DNA, 78 bp, artificial sequence
  Unique molecular identifier - random sequence
  misc_feature (41)..(42): n is a or g or c or t/u
gtctcgtgggctcggagatgtgtataagagacagcttgtannbaaaaaaaaaaaaaaaaaaaaaaaaaaaaaaaaaaa

SEQ ID NO: 3 - DNA, 77 bp, Artificial Sequence
  Unique molecular identifier-random sequence
  misc_feature (40)..(41): n is a or g or c or t/u
tcgtcggcagcgtcagatgtgtataagagacaggccaatnnbaaaaaaaaaaaaaaaaaaaaaaaaaaaaaaaaaaa

SEQ ID NO: 4 - DNA, 77 bp, Artificial Sequence
  Unique molecular sequence - random
  misc_feature (40)..(41): n is a or g or c or t/u
tcgtcggcagcgtcagatgtgtataagagacagcttgtannbaaaaaaaaaaaaaaaaaaaaaaaaaaaaaaaaaaa

SEQ ID NO: 5 - DNA, 60 bp, Artificial Sequence
  Synthetic oligonucleotide sequence for CBMC profiling
ccttggcacccgagaattccaatcacgbaaaaaaaaaaaaaaaaaaaaaaaaaaaaaaaa

SEQ ID NO: 6 - DNA, 60 bp, Artificial Sequence
  Synthetic oligonucleotide sequence for CMBC profiling
ccttggcacccgagaattccacgatgtbaaaaaaaaaaaaaaaaaaaaaaaaaaaaaaaa

SEQ ID NO: 7 - DNA, 59 bp, Artificial Sequence
  Synthetic oligonucleotide sequence for CMBC profiling
ccttggcaccgagaattccattaggcbaaaaaaaaaaaaaaaaaaaaaaaaaaaaaaaa

SEQ ID NO: 8 - DNA, 60 bp, Artificial Sequence
  Synthetic oligonucleotide sequence for CMBC profiling
ccttggcacccgagaattccatgaccabaaaaaaaaaaaaaaaaaaaaaaaaaaaaaaaa

SEQ ID NO: 9 - DNA, 60 bp, Artificial Sequence
  Synthetic oligonucleotide sequence  for CBMC profiling
ccttggcacccgagaattccagccaatbaaaaaaaaaaaaaaaaaaaaaaaaaaaaaaaa

SEQ ID NO: 10 - DNA, 60 bp, Artificial Sequence
  Synthetic oligonucleotide sequence for CMBC profiling
ccttggcacccgagaattccagatcagbaaaaaaaaaaaaaaaaaaaaaaaaaaaaaaaa

SEQ ID NO: 11 - DNA, 60 bp, Artificial Sequence
  Synthetic oligonucleotide sequence for CMBC profiling
ccttggcacccgagaattccatagcttbaaaaaaaaaaaaaaaaaaaaaaaaaaaaaaaa

SEQ ID NO: 12 - DNA, 60 bp, Artificial Sequence
  Synthetic oligonucleotide sequence for CMBC profiling
ccttggcacccgagaattccacttgtabaaaaaaaaaaaaaaaaaaaaaaaaaaaaaaaa

SEQ ID NO: 13 - DNA, 60 bp, Artificial Sequence
  Synthetic oligonucleotide sequence for CMBC profiling
ccttggcacccgagaattccaacttgabaaaaaaaaaaaaaaaaaaaaaaaaaaaaaaaa

SEQ ID NO: 14 - DNA, 60 bp, Artificial Sequence
  Synthetic oligonucleotide sequence for CMBC profiling
ccttggcacccgagaattccaggctacbaaaaaaaaaaaaaaaaaaaaaaaaaaaaaaaa

SEQ ID NO: 15 - DNA, 60 bp, Artificial Sequence
  Synthetic oligonucleotide sequence for CMBC profiling
ccttggcacccgagaattccaagtcaabaaaaaaaaaaaaaaaaaaaaaaaaaaaaaaaa

SEQ ID NO: 16 - DNA, 57 bp, Artificial Sequence
  Synthetic oligonucleotide sequence for CMBC profiling
ccttggcacccgagaattccaagttccbaaaaaaaaaaaaaaaaaaaaaaaaaaaaa

SEQ ID NO: 17 - DNA, 63 bp, Artificial Sequence
  Synthetic oligonucleotide sequence for CMBC profiling
ccttggcacccgagaattccaacagtgbaaaaaaaaaaaaaaaaaaaaaaaaaaaaaaaaaaa

SEQ ID NO: 18 - DNA, 21 bp, Artificial Sequence
  Synthetic oligonucleotide sequence amplification handle
ccttggcacccgagaattcca

SEQ ID NO: 19 - DNA, 21 bp, Artificial Sequence
  Synthetic oligonucleotide sequence amplification handle
ccttggcacccgagaattcca

SEQ ID NO: 20 - DNA, 10 bp, Artificial Sequence
  Synthetic barcode sequence
ttcgtgaggt

SEQ ID NO: 21 - DNA, 10 bp, Artificial Sequence
  Synthetic barcode sequence
tcttcgtcca

SEQ ID NO: 22 - DNA, 10 bp, Artificial Sequence
  Synthetic barcode sequence
atgctctacc

SEQ ID NO: 23 - DNA, 10 bp, Artificial Sequence
  Synthetic barcode sequence
tagacagctg

SEQ ID NO: 24 - DNA, 10 bp, Artificial Sequence
  Synthetic barcode sequence
atggaggtag

SEQ ID NO: 25 - DNA, 10 bp, Artificial Sequence
  Synthetic barcode sequence
agatgaaccc

SEQ ID NO: 26 - DNA, 12 bp, Artificial Sequence
  Synthetic barcode sequence
aggaccatccaa

SEQ ID NO: 27 - DNA, 12 bp, Artificial Sequence
  Synthetic barcode sequence
acatgttaccgt

SEQ ID NO: 28 - DNA, 12 bp, Artificial Sequence
  Synthetic barcode sequence
agcttactatcc

SEQ ID NO: 29 - DNA, 12 bp, Artificial Sequence
  Synthetic barcode sequence
tcgataatgcga

SEQ ID NO: 30 - DNA, 12 bp, Artificial Sequence
  Synthetic barcode sequence
gaggctgagcta

SEQ ID NO: 31 - DNA, 12 bp, Artificial Sequence
  Synthetic barcode sequence
gtgtgacgtatt

SEQ ID NO: 32 - DNA, 12 bp, Artificial Sequence
  Synthetic barcode sequence
actgtctaacgg

SEQ ID NO: 33 - DNA, 12 bp, Artificial Sequence
  Synthetic barcode sequence
tatcacatcggt

SEQ ID NO: 34 - DNA, 79 bp, Artificial Sequence
  Synthetic hashtag oligonucleotide sequence
  misc_feature (35)..(46): n is a, t, c, g  from a barcode or index sequence
gtgactggagttcagacgtgtgctcttccgatctnnnnnnnnnnnnbaaaaaaaaaaaaaaaaaaaaaaaaaaaaaaaa

SEQ ID NO: 35 - DNA, 25 bp, Artificial Sequence
  synthetic oligonucleotide sequence of a hashtag additive
  misc_feature (23)..(24): Bases modified by presence of phosphorothioate bond
gtgactggagttcagacgtgtgctc

SEQ ID NO: 36 - DNA, 20 bp, Artificial Sequence
  Synthetic ADT additive oligonucleotide sequence
  misc_feature (18)..(19): Bases modified by phosphorothioate bond
ccttggcacccgagaattcc

SEQ ID NO: 37 - DNA, 49 bp, Artificial Sequence
  Synthetic PCR oligonucleotide sequence
  misc_feature (47)..(48): Bases modified by phosphorothioate bond
aatgatacggcgaccaccgagatctacactctttccctacacgacgctc

SEQ ID NO: 38 - DNA, 65 bp, Artificial Sequence
  Synthetic oligonucleotide sequence
  misc_feature (25)..(32): n is A, T, G, or C from a barcode or index sequence
  misc_feature (63)..(64): Bases modified by phosphorothioate bond
caagcagaagacggcatacgagatnnnnnnnngtgactggagttccttggcacccgagaattcca

SEQ ID NO: 39 - DNA, 55 bp, Artificial Sequence
  Synthetic sequences forming a hashtag library of primers
  misc_feature (25)..(32): n is A or C or T or G forming a barcode or index sequence
  misc_feature (53)..(54): Bases modified by phosphorothioate bond
caagcagaagacggcatacgagatnnnnnnnngtgactggagttcagacgtgtgc